European Patent Application EP 4 480 959 A1, published December 25, 2024. Title: Novel variant of sigma 38 and method for preparing L-aromatic amino acid using the same. Applicant: DAESANG CORPORATION. The sequence listing filed with the application follows.

SEQUENCE LISTING (24 sequences)

SEQ ID NO: 1 - protein, 132 aa, synthetic construct
MSQNTLKVHDLNEDAEFDENGVEVFDEKALVELEPSDNDLAEEELLSQGATQRVLDATQLYLGEIGYSPLLTAEEEVYFARRALRGDVASRRRMIESNLRLVVKIARRYGNRGLALLDLIEEGNLGLIRAVE

SEQ ID NO: 2 - DNA, 993 bp, synthetic construct
  source 1..993: mol_type = other DNA
atgagtcagaatacgctgaaagttcatgatttaaatgaagatgcggaatttgatgagaacggagttgaggtttttgacgaaaaggccttagtagaattggaacccagtgataacgatttggccgaagaggaactgttatcgcagggagccacacagcgtgtgttggacgcgactcagctttaccttggtgagattggttattcaccactgttaacggccgaagaagaagtttattttgcgcgtcgcgcactgcgtggagatgtcgcctctcgccgccggatgatcgagagtaacttgcgtctggtggtaaaaattgcccgccgttatggcaatcgtggtctggcgttgctggaccttatcgaagagggcaacctggggctgatccgcgcggtagagaagtttgacccggaacgtggtttccgcttctcaacatacgcaacctggtggattcgccagacgattgaacgggcgattatgaaccaaacccgtactattcgtttgccgattcacatcgtaaaggagctgaacgtttacctgcgaaccgcacgtgagttgtcccataagctggaccatgaaccaagtgcggaagagatcgcagagcaactggataagccagttgatgacgtcagccgtatgcttcgtcttaacgagcgcattacctcggtagacaccccgctgggtggtgattccgaaaaagcgttgctggacatcctggccgatgaaaaagagaacggtccggaagataccacgcaagatgacgatatgaagcagagcatcgtcaaatggctgttcgagctgaacgccaaacagcgtgaagtgctggcacgtcgattcggtttgctggggtacgaagcggcaacactggaagatgtaggtcgtgaaattggcctcacccgtgaacgtgttcgccagattcaggttgaaggcctgcgccgtttgcgcgaaatcctgcaaacgcaggggctgaatatcgaagcgctgttccgcgagtaa

SEQ ID NO: 3 - protein, 330 aa, Escherichia coli
MSQNTLKVHDLNEDAEFDENGVEVFDEKALVEQEPSDNDLAEEELLSQGATQRVLDATQLYLGEIGYSPLLTAEEEVYFARRALRGDVASRRRMIESNLRLVVKIARRYGNRGLALLDLIEEGNLGLIRAVEKFDPERGFRFSTYATWWIRQTIERAIMNQTRTIRLPIHIVKELNVYLRTARELSHKLDHEPSAEEIAEQLDKPVDDVSRMLRLNERITSVDTPLGGDSEKALLDILADEKENGPEDTTQDDDMKQSIVKWLFELNAKQREVLARRFGLLGYEAATLEDVGREIGLTRERVRQIQVEGLRRLREILQTQGLNIEALFRE

SEQ ID NO: 4 - DNA, 993 bp, Escherichia coli
  source 1..993: mol_type = genomic DNA
atgagtcagaatacgctgaaagttcatgatttaaatgaagatgcggaatttgatgagaacggagttgaggtttttgacgaaaaggccttagtagaacaggaacccagtgataacgatttggccgaagaggaactgttatcgcagggagccacacagcgtgtgttggacgcgactcagctttaccttggtgagattggttattcaccactgttaacggccgaagaagaagtttattttgcgcgtcgcgcactgcgtggagatgtcgcctctcgccgccggatgatcgagagtaacttgcgtctggtggtaaaaattgcccgccgttatggcaatcgtggtctggcgttgctggaccttatcgaagagggcaacctggggctgatccgcgcggtagagaagtttgacccggaacgtggtttccgcttctcaacatacgcaacctggtggattcgccagacgattgaacgggcgattatgaaccaaacccgtactattcgtttgccgattcacatcgtaaaggagctgaacgtttacctgcgaaccgcacgtgagttgtcccataagctggaccatgaaccaagtgcggaagagatcgcagagcaactggataagccagttgatgacgtcagccgtatgcttcgtcttaacgagcgcattacctcggtagacaccccgctgggtggtgattccgaaaaagcgttgctggacatcctggccgatgaaaaagagaacggtccggaagataccacgcaagatgacgatatgaagcagagcatcgtcaaatggctgttcgagctgaacgccaaacagcgtgaagtgctggcacgtcgattcggtttgctggggtacgaagcggcaacactggaagatgtaggtcgtgaaattggcctcacccgtgaacgtgttcgccagattcaggttgaaggcctgcgccgtttgcgcgaaatcctgcaaacgcaggggctgaatatcgaagcgctgttccgcgagtaa

SEQ ID NO: 5 - DNA, 30 bp, synthetic construct
  source 1..30: mol_type = other DNA
caattttattatagtaattgactattatac

SEQ ID NO: 6 - DNA, 40 bp, synthetic construct
  source 1..40: mol_type = other DNA
ggaacccagtcaattttattatagtaattgactattatac

SEQ ID NO: 7 - DNA, 40 bp, synthetic construct
  source 1..40: mol_type = other DNA
actgggttcctgttctactagttttagagctagaaatagc

SEQ ID NO: 8 - DNA, 30 bp, synthetic construct
  source 1..30: mol_type = other DNA
tgttctactagttttagagctagaaatagc

SEQ ID NO: 9 - DNA, 21 bp, synthetic construct
  source 1..21: mol_type = other DNA
gagcctgtcggcctacctgct

SEQ ID NO: 10 - DNA, 20 bp, synthetic construct
  source 1..20: mol_type = other DNA
cggccggcatgagcctgtcg

SEQ ID NO: 11 - DNA, 30 bp, synthetic construct
  source 1..30: mol_type = other DNA
atgccggccgggtccgggaacaacaagaag

SEQ ID NO: 12 - DNA, 20 bp, synthetic construct
  source 1..20: mol_type = other DNA
ggtccgggaacaacaagaag

SEQ ID NO: 13 - DNA, 20 bp, synthetic construct
  source 1..20: mol_type = other DNA
gccttttcgtcaaaaacctc

SEQ ID NO: 14 - DNA, 30 bp, synthetic construct
  source 1..30: mol_type = other DNA
ttctactaaggccttttcgtcaaaaacctc

SEQ ID NO: 15 - DNA, 30 bp, synthetic construct
  source 1..30: mol_type = other DNA
cttagtagaattggaacccagtgataacga

SEQ ID NO: 16 - DNA, 20 bp, synthetic construct
  source 1..20: mol_type = other DNA
ttggaacccagtgataacga

SEQ ID NO: 17 - DNA, 20 bp, synthetic construct
  source 1..20: mol_type = other DNA
cggatcagccccaggttgcc

SEQ ID NO: 18 - DNA, 20 bp, synthetic construct
  source 1..20: mol_type = other DNA
ctctaccgcgcggatcagcc

SEQ ID NO: 19 - DNA, 33 bp, synthetic construct
  source 1..33: mol_type = other DNA
cgcggtagaggagctcctgaaaatctcgataac

SEQ ID NO: 20 - DNA, 23 bp, synthetic construct
  source 1..23: mol_type = other DNA
gagctcctgaaaatctcgataac

SEQ ID NO: 21 - DNA, 20 bp, synthetic construct
  source 1..20: mol_type = other DNA
ggccgcgttgtttatgctgg

SEQ ID NO: 22 - DNA, 20 bp, synthetic construct
  source 1..20: mol_type = other DNA
ctggtgcgtatgggcggtaa

SEQ ID NO: 23 - DNA, 3234 bp, synthetic construct
  source 1..3234: mol_type = other DNA
tttccataggctccgcccccctgacgagcatcacaaaaatcgacgctcaagtcagaggtggcgaaacccgacaggactataaagataccaggcgtttccccctggaagctccctcgtgcgctctcctgttccgaccctgccgcttaccggatacctgtccgcctttctcccttcgggaagcgtggcgctttctcatagctcacgctgtaggtatctcagttcggtgtaggtcgttcgctccaagctgggctgtgtgcacgaaccccccgttcagcccgaccgctgcgccttatccggtaactatcgtcttgagtccaacccggtaagacacgacttatcgccactggcagcagccactggtaacaggattagcagagcgaggtatgtaggcggtgctacagagttcttgaagtggtggcctaactacggctacactagaaggacagtatttggtatctgcgctctgctgaagccagttaccttcggaaaaagagttggtagctcttgatccggcaaacaaaccaccgctggtagcggtggtttttttgtttgcaagcagcagattacgcgcagaaaaaaaggatctcaagaagatcctttgatcttttctacggggtctgacgctcagtggaacgaaaactcacgttaagggattttggtcatgagattatcaaaaaggatcttcacctagatccttttaaattaaaaatgaagttttaaatcaatctaaagtatatatgagtaaacttggtctgacagttaaaagattgacagtataatagtcaattactataataaaattgatgcgcaggtgaaacacctgctgcagttttagagctagaaatagcaagttaaaataaggctagtccgttatcaacttgaaaaagtggcaccgagtcggtgctttttttcgttttccgggacgccctcgcggacgtgctcatagtccacgacgcccgtgattttgtagccctggccgacggccagcaggtaggccgacaggctcatgccggccggagctcctgaaaatctcgataactcaaaaaatacgcccggtagtgatcttatttcattatggtgaaagttggaacctcttaggatcctctagatttaagaaggagatatacataaaactccttctgagctagttctctagcattctattattttgattcgacaccttaataatagcagaaggagtttttacctgtcaaagaaccatcaaacccttgatacacaaggctttgacctaattttgaaaaatgatgttgtttctatatagtatcaagataagaaagaaaaggatttttcgctacgctcaaatcctttcccgtcacgggcttctcagggcgttttatggcgggtctgctatgtggtgctatctgactttttgctgttcagcagttcctgccctctgattttccagtctgaccacttcggattatcccgtgacaggtcattcagactggctaatgcacccagtaaggcagcggtatcatcaacggggtctgacgctcagtggaacgaaaactcacgttaagggattttggtcatgagattatcaaaaaggatcttcacctagatccttttaaattaaaaatgaagttttaaatcaatctaaagtatatatgagtaaacttggtctgacagttaccaatgcttaatcagtgaggcacctatctcagcgatctgtctatttcgttcatccatagttgcctgactccccgtcgtgtagataactacgatacgggagggcttaccatctggccccagtgctgcaatgataccgcgagacccacgctcaccggctccagatttatcagcaataaaccagccagccggaagggccgagcgcagaagtggtcctgcaactttatccgcctccatccagtctattaattgttgccgggaagctagagtaagtagttcgccagttaatagtttgcgcaacgttgttgccattgctacaggcatcgtggtgtcacgctcgtcgtttggtatggcttcattcagctccggttcccaacgatcaaggcgagttacatgatcccccatgttgtgcaaaaaagcggttagctccttcggtcctccgatcgttgtcagaagtaagttggccgcagtgttatcactcatggttatggcagcactgcataattctcttactgtcatgccatccgtaagatgcttttctgtgactggtgagtactcaaccaagtcattctgagaatagtgtatgcggcgaccgagttgctcttgcccggcgtcaatacgggataataccgcgccacatagcagaactttaaaagtgctcatcattggaaaacgttcttcggggcgaaaactctcaaggatcttaccgctgttgagatccagttcgatgtaacccactcgtgcacccaactgatcttcagcatcttttactttcaccagcgtttctgggtgagcaaaaacaggaaggcaaaatgccgcaaaaaagggaataagggcgacacggaaatgttgaatactcatactcttcctttttcaatattattgaagcatttatcagggttattgtctcatgagcggatacatatttgaatgtatttagaaaaataaacaaataggggttccgcgcacatttccccgaaaagtgccaccaaaaaaacacaaaagaccacattttttaatgtggtctttattcttcaactaaagcacccattagttcaacaaacgaaaattggataaagtgggatatttttaaaatatatatttatgttacagtaagctgcctcgcgcgtttcggtgatgacggtgaaaacctctgacacatgcagctcccggagacggtcacagcttgtctgtaagcggatgccgggagcagacaagcccgtcagggcgcgtcagcgggtgttggcgggtgtcggggcgcagccatgacccagtcacgtagcgatagcggagtgtatactggcttaactatgcggcatcagagcagattgtactgagagtgcaccatatgcggtgtgaaataccgcacagatgcgtaaggagaaaataccgcatcaggcgctcttccgcttcctcgctcactgactcgctgcgctcggtcgttcggctgcggcgagcggtatcagctcactcaaaggcggtaatacggttatccacagaatcaggggataacgcaggaaagaacatgtgagcaaaaggccagcaaaaggccaggaaccgtaaaaaggccgcgttgctggcgtt

SEQ ID NO: 24 - DNA, 9656 bp, synthetic construct
  source 1..9656: mol_type = other DNA
aaagccatgacaaaaacgcgtaacaaaagtgtctataatcacggcagaaaagtccacattgattatttgcacggcgtcacactttgctatgccatagcatttttatccataagattagcggatcctacctgacgctttttatcgcaactctctactgtttctccatacccgtttttttgggaattcgagctctaaggaggttataaaaaatggatattaatactgaaactgagatcaagcaaaagcattcactaaccccctttcctgttttcctaatcagcccggcatttcgcgggcgatattttcacagctatttcaggagttcagccatgaacgcttattacattcaggatcgtcttgaggctcagagctgggcgcgtcactaccagcagctcgcccgtgaagagaaagaggcagaactggcagacgacatggaaaaaggcctgccccagcacctgtttgaatcgctatgcatcgatcatttgcaacgccacggggccagcaaaaaatccattacccgtgcgtttgatgacgatgttgagtttcaggagcgcatggcagaacacatccggtacatggttgaaaccattgctcaccaccaggttgatattgattcagaggtataaaacgaatgagtactgcactcgcaacgctggctgggaagctggctgaacgtgtcggcatggattctgtcgacccacaggaactgatcaccactcttcgccagacggcatttaaaggtgatgccagcgatgcgcagttcatcgcattactgatcgttgccaaccagtacggccttaatccgtggacgaaagaaatttacgcctttcctgataagcagaatggcatcgttccggtggtgggcgttgatggctggtcccgcatcatcaatgaaaaccagcagtttgatggcatggactttgagcaggacaatgaatcctgtacatgccggatttaccgcaaggaccgtaatcatccgatctgcgttaccgaatggatggatgaatgccgccgcgaaccattcaaaactcgcgaaggcagagaaatcacggggccgtggcagtcgcatcccaaacggatgttacgtcataaagccatgattcagtgtgcccgtctggccttcggatttgctggtatctatgacaaggatgaagccgagcgcattgtcgaaaatactgcatacactgcagaacgtcagccggaacgcgacatcactccggttaacgatgaaaccatgcaggagattaacactctgctgatcgccctggataaaacatgggatgacgacttattgccgctctgttcccagatatttcgccgcgacattcgtgcatcgtcagaactgacacaggccgaagcagtaaaagctcttggattcctgaaacagaaagccgcagagcagaaggtggcagcatgacaccggacattatcctgcagcgtaccgggatcgatgtgagagctgtcgaacagggggatgatgcgtggcacaaattacggctcggcgtcatcaccgcttcagaagttcacaacgtgatagcaaaaccccgctccggaaagaagtggcctgacatgaaaatgtcctacttccacaccctgcttgctgaggtttgcaccggtgtggctccggaagttaacgctaaagcactggcctggggaaaacagtacgagaacgacgccagaaccctgtttgaattcacttccggcgtgaatgttactgaatccccgatcatctatcgcgacgaaagtatgcgtaccgcctgctctcccgatggtttatgcagtgacggcaacggccttgaactgaaatgcccgtttacctcccgggatttcatgaagttccggctcggtggtttcgaggccataaagtcagcttacatggcccaggtgcagtacagcatgtgggtgacgcgaaaaaatgcctggtactttgccaactatgacccgcgtatgaagcgtgaaggcctgcattatgtcgtgattgagcgggatgaaaagtacatggcgagttttgacgagatcgtgccggagttcatcgaaaaaatggacgaggcactggctgaaattggttttgtatttggggagcaatggcgatgagatctaaagaggagaaaggatctatggataagaaatactcaataggcttagatatcggcacaaatagcgtcggatgggcggtgatcactgatgaatataaggttccgtctaaaaagttcaaggttctgggaaatacagaccgccacagtatcaaaaaaaatcttataggggctcttttatttgacagtggagagacagcggaagcgactcgtctcaaacggacagctcgtagaaggtatacacgtcggaagaatcgtatttgttatctacaggagattttttcaaatgagatggcgaaagtagatgatagtttctttcatcgacttgaagagtcttttttggtggaagaagacaagaagcatgaacgtcatcctatttttggaaatatagtagatgaagttgcttatcatgagaaatatccaactatctatcatctgcgaaaaaaattggtagattctactgataaagcggatttgcgcttaatctatttggccttagcgcatatgattaagtttcgtggtcattttttgattgagggagatttaaatcctgataatagtgatgtggacaaactatttatccagttggtacaaacctacaatcaattatttgaagaaaaccctattaacgcaagtggagtagatgctaaagcgattctttctgcacgattgagtaaatcaagacgattagaaaatctcattgctcagctccccggtgagaagaaaaatggcttatttgggaatctcattgctttgtcattgggtttgacccctaattttaaatcaaattttgatttggcagaagatgctaaattacagctttcaaaagatacttacgatgatgatttagataatttattggcgcaaattggagatcaatatgctgatttgtttttggcagctaagaatttatcagatgctattttactttcagatatcctaagagtaaatactgaaataactaaggctcccctatcagcttcaatgattaaacgctacgatgaacatcatcaagacttgactcttttaaaagctttagttcgacaacaacttccagaaaagtataaagaaatcttttttgatcaatcaaaaaacggatatgcaggttatattgatgggggagctagccaagaagaattttataaatttatcaaaccaattttagaaaaaatggatggtactgaggaattattggtgaaactaaatcgtgaagatttgctgcgcaagcaacggacctttgacaacggctctattccccatcaaattcacttgggtgagctgcatgctattttgagaagacaagaagacttttatccatttttaaaagacaatcgtgagaagattgaaaaaatcttgacttttcgaattccttattatgttggtccattggcgcgtggcaatagtcgttttgcatggatgactcggaagtctgaagaaacaattaccccatggaattttgaagaagttgtcgataaaggtgcttcagctcaatcatttattgaacgcatgacaaactttgataaaaatcttccaaatgaaaaagtactaccaaaacatagtttgctttatgagtattttacggtttataacgaattgacaaaggtcaaatatgttactgaaggaatgcgaaaaccagcatttctttcaggtgaacagaagaaagccattgttgatttactcttcaaaacaaatcgaaaagtaaccgttaagcaattaaaagaagattatttcaaaaaaatagaatgttttgatagtgttgaaatttcaggagttgaagatagatttaatgcttcattaggtacctaccatgatttgctaaaaattattaaagataaagattttttggataatgaagaaaatgaagatatcttagaggatattgttttaacattgaccttatttgaagatagggagatgattgaggaaagacttaaaacatatgctcacctctttgatgataaggtgatgaaacagcttaaacgtcgccgttatactggttggggacgtttgtctcgaaaattgattaatggtattagggataagcaatctggcaaaacaatattagattttttgaaatcagatggttttgccaatcgcaattttatgcagctgatccatgatgatagtttgacatttaaagaagacattcaaaaagcacaagtgtctggacaaggcgatagtttacatgaacatattgcaaatttagctggtagccctgctattaaaaaaggtattttacagactgtaaaagttgttgatgaattggtcaaagtaatggggcggcataagccagaaaatatcgttattgaaatggcacgtgaaaatcagacaactcaaaagggccagaaaaattcgcgagagcgtatgaaacgaatcgaagaaggtatcaaagaattaggaagtcagattcttaaagagcatcctgttgaaaatactcaattgcaaaatgaaaagctctatctctattatctccaaaatggaagagacatgtatgtggaccaagaattagatattaatcgtttaagtgattatgatgtcgatcacattgttccacaaagtttccttaaagacgattcaatagacaataaggtcttaacgcgttctgataaaaatcgtggtaaatcggataacgttccaagtgaagaagtagtcaaaaagatgaaaaactattggagacaacttctaaacgccaagttaatcactcaacgtaagtttgataatttaacgaaagctgaacgtggaggtttgagtgaacttgataaagctggttttatcaaacgccaattggttgaaactcgccaaatcactaagcatgtggcacaaattttggatagtcgcatgaatactaaatacgatgaaaatgataaacttattcgagaggttaaagtgattaccttaaaatctaaattagtttctgacttccgaaaagatttccaattctataaagtacgtgagattaacaattaccatcatgcccatgatgcgtatctaaatgccgtcgttggaactgctttgattaagaaatatccaaaacttgaatcggagtttgtctatggtgattataaagtttatgatgttcgtaaaatgattgctaagtctgagcaagaaataggcaaagcaaccgcaaaatatttcttttactctaatatcatgaacttcttcaaaacagaaattacacttgcaaatggagagattcgcaaacgccctctaatcgaaactaatggggaaactggagaaattgtctgggataaagggcgagattttgccacagtgcgcaaagtattgtccatgccccaagtcaatattgtcaagaaaacagaagtacagacaggcggattctccaaggagtcaattttaccaaaaagaaattcggacaagcttattgctcgtaaaaaagactgggatccaaaaaaatatggtggttttgatagtccaacggtagcttattcagtcctagtggttgctaaggtggaaaaagggaaatcgaagaagttaaaatccgttaaagagttactagggatcacaattatggaaagaagttcctttgaaaaaaatccgattgactttttagaagctaaaggatataaggaagttaaaaaagacttaatcattaaactacctaaatatagtctttttgagttagaaaacggtcgtaaacggatgctggctagtgccggagaattacaaaaaggaaatgagctggctctgccaagcaaatatgtgaattttttatatttagctagtcattatgaaaagttgaagggtagtccagaagataacgaacaaaaacaattgtttgtggagcagcataagcattatttagatgagattattgagcaaatcagtgaattttctaagcgtgttattttagcagatgccaatttagataaagttcttagtgcatataacaaacatagagacaaaccaatacgtgaacaagcagaaaatattattcatttatttacgttgacgaatcttggagctcccgctgcttttaaatattttgatacaacaattgatcgtaaacgatatacgtctacaaaagaagttttagatgccactcttatccatcaatccatcactggtctttatgaaacacgcattgatttgagtcagctaggaggtgactaacgcatcctcacgataatatccgggtaggcgcaatcactttcgtctactccgttacaaagcgaggctgggtatttcccggcctttctgttatccgaaatccactgaaagcacagcggctggctgaggagataaataataaacgaggggctgtatgcacaaagcatcttctgttgagttaagaacgagtatcgagatggcacatagccttgctcaaattggaatcaggtttgtgccaataccagtagaaacagacgaagaatccatgggtatggacagttttccctttgatatgtaacggtgaacagttgttctacttttgtttgttagtcttgatgcttcactgatagatacaagagccaaatctagtaatattttatctgattaataagatgatcttcttgagatcgttttggtctgcgcgtaatctcttgctctgaaaacgaaaaaaccgccttgcagggcggtttttcgaaggttctctgagctaccaactctttgaaccgaggtaactggcttggaggagcgcagtcaccaaaacttgtcctttcagtttagccttaaccggcgcatgacttcaagactaactcctctaaatcaattaccagtggctgctgccagtggtgcttttgcatgtctttccgggttggactcaagacgatagttaccggataaggcgcagcggtcggactgaacggggggttcgtgcatacagtccagcttggagcgaactgcctacccggaactgagtgtcaggcgtggaatgagacaaacgcggccataacagcggaatgacaccggtaaaccgaaaggcaggaacaggagagcgcacgagggagccgccagggggaaacgcctggtatctttatagtcctgtcgggtttcgccaccactgatttgagcgtcagatttcgtgatgcttgtcaggggggcggagcctatggaaaaacggctttgccgcggccccgctgaatattccttttgtctccgaccatcaggcacctgagtcgctgtctttttcgtgacattcagttcgctgcgctcacggctctggcagtgaatgggggtaaatggcactacaggcgccttttatggattcatgcaaggaaactacccataatacaagaaaagatgtggtctttattcttcaactaaagcacccattagttcaacaaacgaaaattggataaagtgggatatttttaaaatatatatttatgttacctggcagagcctgtactttttacagtcggttttctaatgtcactaacctgccccgttagtcgccatttgcatcgatttattatgacaacttgacggctacatcattcactttttcttcacaaccggcacggaactcgctcgggctggccccggtgcattttttaaatacccgcgagaaatagagttgatcgtcaaaaccaacattgcgaccgacggtggcgataggcatccgggtggtgctcaaaagcagcttcgcctggctgatacgttggtcctcgcgccagcttaagacgctaatccctaactgctggcggaaaagatgtgacagacgcgacggcgacaagcaaacatgctgtgcgacgctggcgatatcaaaattgctgtctgccaggtgatcgctgatgtactgacaagcctcgcgtacccgattatccatcggtggatggagcgactcgttaatcgcttccatgcgccgcagtaacaattgctcaagcagatttatcgccagcagctccgaatagcgcccttccccttgcccggcgttaatgatttgcccaaacaggtcgctgaaatgcggctggtgcgcttcatccgggcgaaagaaccccgtattggcaaatattgacggccagttaagccattcatgccagtaggcgcgcggacgaaagtaaacccactggtgataccattcgcgagcctccggatgacgaccgtagtgatgaatctctcctggcgggaacagcaaaatatcacccggtcggcaaacaaattctcgtccctgatttttcaccaccccctgaccgcgaatggtgagattgagaatataacctttcattcccagcggtcggtcgataaaaaaatcgagataaccgttggcctcaatcggcgttaaacccgccaccagatgggcattaaacgagtatcccggcagcaggggatcattttgcgcttcagccatacttttcatactcccgccattcagagaagaaaccaattgtccatattgcatcagacattgccgtcactgcgtcttttactggctcttctcgctaaccaaaccggtaaccccgcttattaaaagcattctgtaacaaagcgggaccagtaatagaaagtgagggagccacggttgatgagagctttgttgtaggtggaccagttggtgattttgaacttttgctttgccacggaacggtctgcgttgtcgggaagatgcgtgatctgatccttcaactcagcaaaagttcgatttattcaacaaagccacgttgtgtctcaaaatctctgatgttacattgcacaagataaaaatatatcatcatgaacaataaaactgtctgcttacataaacagtaatacaaggggtgttatgagccatattcaacgggaaacgtcttgctcgaggccgcgattaaattccaacatggatgctgatttatatgggtataaatgggctcgcgataatgtcgggcaatcaggtgcgacaatctatcgattgtatgggaagcccgatgcgccagagttgtttctgaaacatggcaaaggtagcgttgccaatgatgttacagatgagatggtcagactaaactggctgacggaatttatgcctcttccgaccatcaagcattttatccgtactcctgatgatgcatggttactcaccactgcgatccccgggaaaacagcattccaggtattagaagaatatcctgattcaggtgaaaatattgttgatgcgctggcagtgttcctgcgccggttgcattcgattcctgtttgtaattgtccttttaacagcgatcgcgtatttcgtctcgctcaggcgcaatcacgaatgaataacggtttggttgatgcgagtgattttgatgacgagcgtaatggctggcctgttgaacaagtctggaaagaaatgcataagcttttgccattctcaccggattcagtcgtcactcatggtgatttctcacttgataaccttatttttgacgaggggaaattaataggttgtattgatgttggacgagtcggaatcgcagaccgataccaggatcttgccatcctatggaactgcctcggtgagttttctccttcattacagaaacggctttttcaaaaatatggtattgataatcctgatatgaataaattgcagtttcatttgatgctcgatgagtttttctaatcagaattggttaattggttgtaaca